European Patent Application EP 4 559 938 A1, published May 28, 2025. Title: 一种抗组织因子人源化抗体及制备的抗体偶联药物和应用. Applicant: 山西纳安生物科技股份有限公司. Application CN. The sequence listing filed with the application follows.

SEQUENCE LISTING (49 sequences)

SEQ ID NO: 1 - protein, 449 aa, unidentified
QIQLVQSGPEVVKPGASVRVSCKGSGYSFTDYNIYWVRQSPAKGLEWIGYIDPYNGLTIYDQNFRAKATLSVDHSTSNAYMEINSLRYEDTAVYFCARDVTSALEFWGQGTSVTVSSEFASTKGPSVFPLAPSSKSTSGGTAALGCLVKDYFPEPVTVSWNSGALTSGVHTFPAVLQSSGLYSLSSVVTVPSSSLGTQTYICNVNHKPSNTKVDKKVEPKSCDKTHTCPPCPAPELLGGPSVFLFPPKPKDTLMISRTPEVTCVVVDVSHEDPEVKFNWYVDGVEVHNAKTKPREEQYNSTYRVVSVLTVLHQDWLNGKEYKCKVSNKALPAPIEKTISKAKGQPREPQVYTLPPSRDELTKNQVSLTCLVKGFYPSDIAVEWESNGQPENNYKTTPPVLDSDGSFFLYSKLTVDKSRWQQGNVFSCSVMHEALHNHYTQKSLSLSPGK

SEQ ID NO: 2 - protein, 214 aa, synthetic construct
DIQMTQSPASISASVGERVTITCLGSQTIDTYLAWYLQKPGRSPQLLIYAATQLADGVPSRFSASGSGTDFSLTISSLQPEDVATYYCQNVYSSPFTFGQGNKLEIKRTVAAPSVFIFPPSDEQLKSGTASVVCLLNNFYPREAKVQWKVDNALQSGNSQESVTEQDSKDSTYSLSSTLTLSKADYEKHKVYACEVTHQGLSSPVTKSFNRGEC

SEQ ID NO: 3 - protein, 449 aa, unidentified
QIQLVQSGPELVKPGASVQVSCKTSGYSFTDYNVYWVRQSPAKGIEWIGYIDPYNGLTIYEQNFRGKGTLSLDHSTSTAYMELNSLRYEDTAVYFCARDVTTALDFWGQGTSVTVSSEFASTKGPSVFPLAPSSKSTSGGTAALGCLVKDYFPEPVTVSWNSGALTSGVHTFPAVLQSSGLYSLSSVVTVPSSSLGTQTYICNVNHKPSNTKVDKKVEPKSCDKTHTCPPCPAPELLGGPSVFLFPPKPKDTLMISRTPEVTCVVVDVSHEDPEVKFNWYVDGVEVHNAKTKPREEQYNSTYRVVSVLTVLHQDWLNGKEYKCKVSNKALPAPIEKTISKAKGQPREPQVYTLPPSRDELTKNQVSLTCLVKGFYPSDIAVEWESNGQPENNYKTTPPVLDSDGSFFLYSKLTVDKSRWQQGNVFSCSVMHEALHNHYTQKSLSLSPGK

SEQ ID NO: 4 - protein, 214 aa, synthetic construct
DIQMTQSPASISASIGERVTITCLASQTIDTWLAWFLQKPGRSPNLLIYAATNLADGVPYRFSASGSGNDFSLTISSLNPEDVATYYCQQVYSSPFTFGQGNKLEIRRTVAAPSVFIFPPSDEQLKSGTASVVCLLNNFYPREAKVQWKVDNALQSGNSQESVTEQDSKDSTYSLSSTLTLSKADYEKHKVYACEVTHQGLSSPVTKSFNRGEC

SEQ ID NO: 5 - protein, 483 aa, synthetic construct
QIQLVQSGPELVKPGASVQVSCKTSGYSFTDYNVYWVRQSPAKGIEWIGYIDPYNGLTIYEQNFRGKGTLSLDHSTSTAYMELNSLRYEDTAVYFCARDVTTALDFWGQGTSVTVSSGGGGSGGGGSGGGGSDIQMTQSPASISASIGERVTITCLASQTIDTWLAWFLQKPGRSPNLLIYAATNLADGVPYRFSASGSGNDFSLTISSLNPEDVATYYCQQVYSSPFTFGQGNKLEIRGGAGGGMSKGEELFTGVVPILVELDGDVNGHKFSVSGEGEGDATYGKLTLKFICTTGKLPVPWPTLVTTFSYGVQCFSRYPDHMKQHDFFKSAMPEGYVQERTIFFKDDGNYKTRAEVKFEGDTLVNRIELKGIDFKEDGNILGHKLEYNYNSHNVYIMADKQKNGIKVNFKIRHNIEDGSVQLADHYQQNTPIGDGPVLLPDNHYLSTQSALSKDPNEKRDHMVLLEFVTAAGITHGMDELYK

SEQ ID NO: 6 - DNA, 1449 bp, synthetic construct
  source 1..1449: mol_type = other DNA
caaatccagctggttcagagcggtccagaactggttaaaccgggcgcttctgtacaggtttcttgcaaaacctccggttactccttcaccgactacaatgtgtactgggttcgccagtctcctgctaaaggcatcgagtggatcggttacatcgacccgtacaacggcctgactatttacgaacagaattttcgtggcaaaggcaccctgtctctggatcattctaccagcaccgcttatatggaactgaatagcctgcgttacgaagataccgcggtttatttctgtgctcgtgatgtaactactgccctggacttttggggccagggtacgtctgtaaccgtaagctctggtggtggcggttctggcggtggtggttctggtggtggtggtagcgatatccagatgacccagtctccggcttccattagcgcctccatcggtgagcgtgtcaccatcacttgcctggccagccagaccatcgatacttggctggcatggttcctgcagaaaccgggtcgtagcccaaatctgctgatctacgctgcaacgaacctggcggacggcgttccgtaccgtttttccgcgtccggctccggtaacgacttcagcctgaccatctcttctctgaaccctgaagatgtcgcaacgtactactgccagcaggtatacagcagcccgttcaccttcggtcagggcaacaaactggagatccgcggtggcgccggtggcggtatgtctaaaggtgaagagctgtttactggtgttgttccgatcctggtggagctggacggtgatgttaacggccataaattcagcgtgtctggtgaaggcgagggtgacgccacctacggtaaactgaccctgaaattcatctgtaccacgggcaaactgccggtaccatggccgacgctggttaccaccttctcctatggtgtgcagtgcttttcccgctacccggaccatatgaaacagcacgatttctttaaaagcgcgatgccggaaggctacgtacaggaacgcactatctttttcaaggacgacggcaactataaaacccgtgcagaagtcaaattcgagggtgacaccctggtcaaccgcatcgaactgaaaggcatcgacttcaaagaggacggtaacatcctgggtcacaaactggaatacaactataactcccacaacgtgtacattatggcggataagcagaaaaacggcattaaagtcaacttcaaaatccgccataacattgaagatggttccgttcagctggccgaccactaccagcagaatactccgatcggtgatggcccggtcctgctgccggataaccactacctgagcacccaatctgctctgtccaaggacccgaacgagaaacgcgaccatatggttctgctggaatttgtaaccgcggcgggtatcactcacggcatggatgaactgtataaa

SEQ ID NO: 7 - protein, 30 aa, synthetic construct
EVQLQQSGPELVKPGASVKVSCKASGYTFT

SEQ ID NO: 8 - protein, 30 aa, synthetic construct
QIQLVQSGPELVKPGASVQVSCKTSGYSFT

SEQ ID NO: 9 - protein, 30 aa, synthetic construct
QIQLVQSGPEVVKPGASVRVSCKGSGYSFT

SEQ ID NO: 10 - protein, 5 aa, synthetic construct
HFNVY

SEQ ID NO: 11 - protein, 5 aa, synthetic construct
DYNVY

SEQ ID NO: 12 - protein, 5 aa, synthetic construct
DYNIY

SEQ ID NO: 13 - protein, 14 aa, synthetic construct
WVRQSPGKGLEWIG

SEQ ID NO: 14 - protein, 14 aa, synthetic construct
WVRQSPAKGIEWIG

SEQ ID NO: 15 - protein, 14 aa, synthetic construct
WVRQSPAKGLEWIG

SEQ ID NO: 16 - protein, 16 aa, synthetic construct
YIDPDNGITFYDENFM

SEQ ID NO: 17 - protein, 16 aa, synthetic construct
YIDPYNGLTIYEQNFR

SEQ ID NO: 18 - protein, 16 aa, synthetic construct
YIDPYNGLTIYDQNFR

SEQ ID NO: 19 - protein, 33 aa, synthetic construct
GKATLTVDKSSSTAYMQLNSLTSEDSAVYYCAR

SEQ ID NO: 20 - protein, 33 aa, synthetic construct
GKGTLSLDHSTSTAYMELNSLRYEDTAVYFCAR

SEQ ID NO: 21 - protein, 33 aa, synthetic construct
AKATLSVDHSTSNAYMEINSLRYEDTAVYFCAR

SEQ ID NO: 22 - protein, 8 aa, synthetic construct
DVTTAVDF

SEQ ID NO: 23 - protein, 8 aa, synthetic construct
DVTTALDF

SEQ ID NO: 24 - protein, 8 aa, synthetic construct
DVTSALEF

SEQ ID NO: 25 - protein, 11 aa, synthetic construct
WGQGTTLTVSS

SEQ ID NO: 26 - protein, 11 aa, synthetic construct
WGQGTSVTVSS

SEQ ID NO: 27 - protein, 23 aa, synthetic construct
DIQMTQSPSSLSASVGDRVTITC

SEQ ID NO: 28 - protein, 23 aa, synthetic construct
DIQMTQSPASISASIGERVTITC

SEQ ID NO: 29 - protein, 23 aa, synthetic construct
DIQMTQSPASISASVGERVTITC

SEQ ID NO: 30 - protein, 11 aa, synthetic construct
LATQTLDTWLA

SEQ ID NO: 31 - protein, 11 aa, synthetic construct
LASQTIDTWLA

SEQ ID NO: 32 - protein, 11 aa, synthetic construct
LGSQTIDTYLA

SEQ ID NO: 33 - protein, 15 aa, synthetic construct
WYQQKPGKAPQLLIY

SEQ ID NO: 34 - protein, 6 aa, synthetic construct
WFLQKP

SEQ ID NO: 35 - protein, 15 aa, synthetic construct
WYLQKPGRSPQLLIY

SEQ ID NO: 36 - protein, 7 aa, synthetic construct
AATYLAD

SEQ ID NO: 37 - protein, 7 aa, synthetic construct
AATNLAD

SEQ ID NO: 38 - protein, 7 aa, synthetic construct
AATQLAD

SEQ ID NO: 39 - protein, 32 aa, synthetic construct
GVPSRFSGSGSGTDFTFTISSLQPEDFATYYC

SEQ ID NO: 40 - protein, 32 aa, synthetic construct
GVPYRFSASGSGNDFSLTISSLNPEDVATYYC

SEQ ID NO: 41 - protein, 32 aa, synthetic construct
GVPSRFSASGSGTDFSLTISSLQPEDVATYYC

SEQ ID NO: 42 - protein, 9 aa, synthetic construct
QLVYSSPST

SEQ ID NO: 43 - protein, 9 aa, synthetic construct
QQVYSSPFT

SEQ ID NO: 44 - protein, 9 aa, synthetic construct
QNVYSSPFT

SEQ ID NO: 45 - protein, 10 aa, synthetic construct
FGQGTKLEIK

SEQ ID NO: 46 - protein, 10 aa, synthetic construct
FGQGNKLEIR

SEQ ID NO: 47 - protein, 117 aa, synthetic construct
QIQLVQSGPELVKPGASVQVSCKTSGYSFTDYNVYWVRQSPAKGIEWIGYIDPYNGLTIYEQNFRGKGTLSLDHSTSTAYMELNSLRYEDTAVYFCARDVTTALDFWGQGTSVTVSS

SEQ ID NO: 48 - protein, 107 aa, synthetic construct
DIQMTQSPASISASIGERVTITCLASQTIDTWLAWFLQKPGRSPNLLIYAATNLADGVPYRFSASGSGNDFSLTISSLNPEDVATYYCQQVYSSPFTFGQGNKLEIR

SEQ ID NO: 49 - protein, 10 aa, synthetic construct
FGQGNKLEIK